European Patent Specification EP 3 768 281 B1, published July 5, 2023. Title: COMPOSITIONS AND METHODS FOR T-CELL AND CYTOKINE ACTIVATION. Applicant: THE REGENTS OF THE UNIVERSITY OF MICHIGAN. The sequence listing filed with the application follows.

SEQUENCE LISTING (14 sequences)

SEQ ID NO: 1 - protein, 459 aa, Homo sapiens [sequence omitted]

SEQ ID NO: 2 - DNA, 72 bp, Homo sapiens
ccaatcctgctgacaatcagcatcctgagctttttcagcgtggccctgctggtcattctggccgtgctgtgg

SEQ ID NO: 3 - DNA, 72 bp, Homo sapiens
ccaatcctgctgataatcagcatcctgagctttttcagcgtggccctgctggtcattctggccgtgctgtgg

SEQ ID NO: 4 - DNA, 585 bp, Homo sapiens
aagaagcggatcaagcctatcgtgtggcccagcctgcctgaccacaaaaagaccctggaacacctgtgcaagaagccccggaagaacctgaacgtgtccttcaatcccgagagcttcctggactgtcagattcacagagtggacgacatccaggccagagatgaggtggaaggctttctgcaggacacattccctcagcagctggaagagagcgagaagcagagactcggcggagatgtgcagtcccctaattgccctagcgaggacgtcgtgatcacccctgagagcttcggcagagatagctccctgacatgtctggccggcaatgtgtccgcctgtgatgcccctatcctgagcagctccagaagcctggattgcagagagagcggcaagaacggccctcacgtgtaccaagatctgctgctgagcctgggcaccaccaattctacactgcctccaccattcagcctgcagagcggcatcctgacactgaaccctgttgctcagggccagccaatcctgacaagcctgggctccaatcaagaagaggcctacgtcaccatgagcagcttctaccagaaccag

SEQ ID NO: 5 - DNA, 48 bp, Homo sapiens
gagcctaagagctgcgataagacccacacctgtcctccatgtcctgat

SEQ ID NO: 6 - DNA, 777 bp, Homo sapiens
atggccacaaccgactggatctggcggatcctgtttcttgtgggagccgccacaggcgcccattctcaggttcaacttcagcagcctggcgccgaactcgttagacctggcgcttctgtgaagctgagctgcaaggccagcggctacaccttcaccagctactggatgaactgggtcaagcagaggcccgaccagggcctcgaatggatcggaagaatcgacccctacgacagcgagacacactacaaccagaagttcaaggacaaggccatcctgaccgtggacaagagcagcagcacagcctacatgcagctgagcagcctgaccagcgaagatagcgccgtgtactactgcgccagaggcaactgggatgactattggggccagggcaccacactgacagtttctagcggaggcggaggttctggtggcggaggaagtggcggcggaggatctgatgtgcagatcacacagagccccagctacctggctgcatctcctggcgagacaatcaccatcaactgccgggccagcaagagcatctccaaggacctggcctggtatcaagagaagcccggcaagaccaacaagctgctgatctacagcggcagcacactgcagtctggcatccccagcagattttccggctctggcagcggcaccgatttcaccctgaccataagctccctggaacctgaggacttcgccatgtactattgccagcagcataacaagtacccgtacaccttcggcggaggcaccaagctcgagatcaag

SEQ ID NO: 7 - DNA, 18 bp, Artificial sequence
  Forward Primer
aagaccctggaacacctg

SEQ ID NO: 8 - DNA, 19 bp, Artificial sequence
  Reverse Primer
gataggcttgatccgcttc

SEQ ID NO: 9 - DNA, 22 bp, Artificial sequence
  Forward Primer
agaagaggccttcgtcaccatg

SEQ ID NO: 10 - DNA, 18 bp, Artificial sequence
  Reverse Primer
tgattggagcccaggctt

SEQ ID NO: 11 - protein, 15 aa, Homo sapiens
KPIVWPSLPNHKKTL

SEQ ID NO: 12 - protein, 6 aa, Homo sapiens
KPIKTL

SEQ ID NO: 13 - protein, 7 aa, Homo sapiens
EEAYVTM

SEQ ID NO: 14 - protein, 7 aa, Homo sapiens
EEAFVTM